European Patent Application EP 4 357 357 A1, published April 24, 2024. Title: HUMAN INTERLEUKIN-2 VARIANT AND USE THEREOF. Applicant: Yunquan Biotechnology (Beijing) Co., Ltd. Application WO PCT/CN2022/105789, filed July 14, 2022. The sequence listing filed with the application follows.

SEQUENCE LISTING (16 sequences)

SEQ ID NO: 1 - protein, 133 aa, Homo sapiens [sequence omitted]

SEQ ID NO: 2 - protein, 130 aa, synthetic construct
  REGION 1..130: note = IL-2-1
APTSSSTKKTQLQLEHLLLDLQMILNGINNGGNPMHGLDGFGMPKKATELKHLQCLEEELKPLEEVLNLAQSKNFHLRPRDLISNINVIVLELKGSETTFMCEYADETATIVEFLNRWITFAQSIISTLT

SEQ ID NO: 3 - protein, 132 aa, synthetic construct
  REGION 1..132: note = IL-2-2
APTSSSTKKTQLQLEHLLLDLQMILNGINNYKNPMHGLDGFKFYMPKKATELKHLQCLEEELKPLEEVLNLAQSKNFHLRPRDLISNINVIVLELKGSETTFMCEYADETATIVEFLNRWITFAQSIISTLT

SEQ ID NO: 4 - protein, 133 aa, synthetic construct
  REGION 1..133: note = IL-2-3
APTSSSTKKTQLQLEHLLLDLQMILNGINNGGNPKLTRMLTFKFYMPKKATELKHLQCLEEELKPLEEVLNLAQSKNFHLRPRDLISNINVIVLELKGSETTFMCEYADETATIVEFLNRWITFAQSIISTLT

SEQ ID NO: 5 - protein, 131 aa, synthetic construct
  REGION 1..131: note = IL-2-4
APTSSSTKKTQLQLEHLLLDLQMILNGINNYKNPKLTRMLTFGMPKKATELKHLQCLEEELKPLEEVLNLAQSKNFHLRPRDLISNINVIVLELKGSETTFMCEYADETATIVEFLNRWITFAQSIISTLT

SEQ ID NO: 6 - protein, 132 aa, synthetic construct
  REGION 1..132: note = IL-2-5
APTSSSTKKTQLQLEHLLLDLQMILNGINNGGNPMHGLDGFKFYMPKKATELKHLQCLEEELKPLEEVLNLAQSKNFHLRPRDLISNINVIVLELKGSETTFMCEYADETATIVEFLNRWITFAQSIISTLT

SEQ ID NO: 7 - protein, 130 aa, synthetic construct
  REGION 1..130: note = IL-2-6
APTSSSTKKTQLQLEHLLLDLQMILNGINNYKNPMHGLDGFGMPKKATELKHLQCLEEELKPLEEVLNLAQSKNFHLRPRDLISNINVIVLELKGSETTFMCEYADETATIVEFLNRWITFAQSIISTLT

SEQ ID NO: 8 - protein, 131 aa, synthetic construct
  REGION 1..131: note = IL-2-7
APTSSSTKKTQLQLEHLLLDLQMILNGINNGGNPKLTRMLTFGMPKKATELKHLQCLEEELKPLEEVLNLAQSKNFHLRPRDLISNINVIVLELKGSETTFMCEYADETATIVEFLNRWITFAQSIISTLT

SEQ ID NO: 9 - protein, 130 aa, synthetic construct
  REGION 1..130: note = IL-2-8
APTSSSTKKTQLQLEHLLLDLQMILNGINNYKNPMGGLGGFYMPKKATELKHLQCLEEELKPLEEVLNLAQSKNFHLRPRDLISNINVIVLELKGSETTFMCEYADETATIVEFLNRWITFAQSIISTLT

SEQ ID NO: 10 - protein, 130 aa, synthetic construct
  REGION 1..130: note = IL-2-9
APTSSSTKKTQLQLEHLLLDLQMILNGINNYKNPGGGGGGFGMPKKATELKHLQCLEEELKPLEEVLNLAQSKNFHLRPRDLISNINVIVLELKGSETTFMCEYADETATIVEFLNRWITFAQSIISTLT

SEQ ID NO: 11 - protein, 12 aa, synthetic construct
GGNPMHGLDGFG

SEQ ID NO: 12 - protein, 6 aa, synthetic construct
MHGLDG

SEQ ID NO: 13 - protein, 6 aa, synthetic construct
MGGLGG

SEQ ID NO: 14 - protein, 6 aa, synthetic construct
GGGGGG

SEQ ID NO: 15 - protein, 362 aa, synthetic construct
  REGION 1..362: note = IL-2-10
APTSSSTKKTQLQLEHLLLDLQMILNGINNGGNPMHGLDGFGMPKKATELKHLQCLEEELKPLEEVLNLAQSKNFHLRPRDLISNINVIVLELKGSETTFMCEYADETATIVEFLNRWITFAQSIISTLTEPKSADKTHTCPPCPAPELLGGPSVFLFPPKPKDTLMISRTPEVTCVVVDVSHEDPEVKFNWYVDGVEVHNAKTKPREEQYNSTYRVVSVLTVLHQDWLNGKEYKCKVSNKALPAPIEKTISKAKGQPREPQVYTLPPSREEMTKNQVSLTCLVKGFYPSDIAVEWESNGQPENNYKTTPPVLDSDGSFFLYSKLTVDKSRWQQGNVFSCSVMHEALHNHYTQKSLSLSPGK

SEQ ID NO: 16 - protein, 232 aa, Homo sapiens
EPKSADKTHTCPPCPAPELLGGPSVFLFPPKPKDTLMISRTPEVTCVVVDVSHEDPEVKFNWYVDGVEVHNAKTKPREEQYNSTYRVVSVLTVLHQDWLNGKEYKCKVSNKALPAPIEKTISKAKGQPREPQVYTLPPSREEMTKNQVSLTCLVKGFYPSDIAVEWESNGQPENNYKTTPPVLDSDGSFFLYSKLTVDKSRWQQGNVFSCSVMHEALHNHYTQKSLSLSPGK